European Patent Application EP 4 276 182 A1, published November 15, 2023. Title: TRANSCRIPTION PRODUCT IN ORGANISM CELLS INCLUDING HUMAN AND GENE-INTRODUCED RNA AND COMPLEX PURIFICATION TOOL THEREOF. Applicant: KAWASAKI GAKUEN EDUCATIONAL FOUNDATION. The sequence listing filed with the application follows.

SEQUENCE LISTING (25 sequences)

SEQ ID NO: 1 - DNA, 310 bp, Artificial Sequence
  crRNA
gagggcctatttcccatgattccttcatatttgcatatacgatacaaggctgttagagagataattagaattaatttgactgtaaacacaaagatattagtacaaaatacgtgacgtagaaagtaataatttcttgggtagtttgcagttttaaaattatgttttaaaatggactatcatatgcttaccgtaacttgaaagtatttcgatttcttggctttatatatcttgtggaaaggacgaaacaccgatttagactaccccaaaaacgaaggggactaaaacggagacgtgaccgtctccttttttt

SEQ ID NO: 2 - DNA, 5228 bp, Artificial Sequence
  dCas13a
accatgaaagtgaccaaggtcgacggcatcagccacaagaagtacatcgaagagggcaagctcgtgaagtccaccagcgaggaaaaccggaccagcgagagactgagcgagctgctgagcatccggctggacatctacatcaagaaccccgacaacgcctccgaggaagagaaccggatcagaagagagaacctgaagaagttctttagcaacaaggtgctgcacctgaaggacagcgtgctgtatctgaagaaccggaaagaaaagaacgccgtgcaggacaagaactatagcgaagaggacatcagcgagtacgacctgaaaaacaagaacagcttctccgtgctgaagaagatcctgctgaacgaggacgtgaactctgaggaactggaaatctttcggaaggacgtggaagccaagctgaacaagatcaacagcctgaagtacagcttcgaagagaacaaggccaactaccagaagatcaacgagaacaacggtacccatactctttatgcccccggtggatatgacattatgggatatctggaccagatcggcaaccggccaaacccgcaggtggaactgggccccgtggatacatcctgcgccttgattctttgtgacctgaaacagaaagacaccccgatagtttacgcgagtgaagccttcctctacatgacaggttacagcaacgcagaggtgctgggccggaattgccggtttctgcaaagccctgacggcatggtgaagcccaagagcacccggaagtacgtggatagtaacacaatcaatactatgcgcaaggcaatcgacaggaatgccgaggtgcaggttgaagtagtcaattttaaaaagaatggacagcgatttgttaatttcctgactatgatacctgttagggacgaaacaggcgagtatcgatactctatgggattccagtgcgaaacagaaggcggaagcggtggcggatccggcagcggcgccaccaacttcagcctgctgaagcaggccggcgacgtggaggagaaccccggccccctcgagggcggacatactctttatgcccccggtggatatgacattatgggatatctgaggcagatcaggaaccggccaaacccgcaggtggaactgggccccgtggatacatcctgcgccttgattctttgtgacctgaaacagaaagacaccccgatagtttacgcgagtgaagccttcctctacatgacaggttacagcaacgcagaggtgctgggccggaattgccggtttctgcaaagccctgacggcatggtgaagcccaagagcacccggaagtacgtggatagtaacacaatcaatactatgcgcaaggcaatcgacaggaatgccgaggtgcaggttgaagtagtcaattttaaaaagaatggacagcgatttgttaatttcctgactatgatacctgttagggacgaaacaggcgagtatcgatactctatgggattccagtgcgaaacagaaggtaccgtggaaaaagtgggcggcaagagcaagcggaacatcatctacgactactacagagagagcgccaagcgcaacgactacatcaacaacgtgcaggaagccttcgacaagctgtataagaaagaggatatcgagaaactgtttttcctgatcgagaacagcaagaagcacgagaagtacaagatccgcgagtactatcacaagatcatcggccggaagaacgacaaagagaacttcgccaagattatctacgaagagatccagaacgtgaacaacatcaaagagctgattgagaagatccccgacatgtctgagctgaagaaaagccaggtgttctacaagtactacctggacaaagaggaactgaacgacaagaatattaagtacgccttctgccacttcgtggaaatcgagatgtcccagctgctgaaaaactacgtgtacaagcggctgagcaacatcagcaacgataagatcaagcggatcttcgagtaccagaatctgaaaaagctgatcgaaaacaaactgctgaacaagctggacacctacgtgcggaactgcggcaagtacaactactatctgcaagtgggcgagatcgccacctccgactttatcgcccggaaccggcagaacgaggccttcctgagaaacatcatcggcgtgtccagcgtggcctacttcagcctgaggaacatcctggaaaccgagaacgagaacggtatcaccggccggatgcggggcaagaccgtgaagaacaacaagggcgaagagaaatacgtgtccggcgaggtggacaagatctacaatgagaacaagcagaacgaagtgaaagaaaatctgaagatgttctacagctacgacttcaacatggacaacaagaacgagatcgaggacttcttcgccaatatcgatgaggccatctctagtattgctcacggcatcgtgcatttcaacctggaactggaaggcaaggacatcttcgccttcaagaatatcgcccccagcgagatctccaagaagatgtttcagaacgaaatcaacgaaaagaagctgaagctgaaaatcttcaagcagctgaacagcgccaacgtgttcaactactacgagaaggatgtgatcatcaagtacctgaagaataccaagttcaacttcgtgaacaaaaacatccccttcgtgcccagcttcaccaagctgtacaacaagattgaggacctgcggaataccctgaagtttttttggagcgtgcccaaggacaaagaagagaaggacgcccagatctacctgctgaagaatatctactacggcgagttcctgaacaagttcgtgaaaaactccaaggtgttctttaagatcaccaatgaagtgatcaagattaacaagcagcggaaccagaaaaccggccactacaagtatcagaagttcgagaacatcgagaaaaccgtgcccgtggaatacctggccatcatccagagcagagagatgatcaacaaccaggacaaagaggaaaagaatacctacatcgactttattcagcagattttcctgaagggcttcatcgactacctgaacaagaacaatctgaagtatatcgagagcaacaacaacaatgacaacaacgacatcttctccaagatcaagatcaaaaaggataacaaagagaagtacgacaagatcctgaagaactatgagaagcacaatcggaacaaagaaatccctcacgagatcaatgagttcgtgcgcgagatcaagctggggaagattctgaagtacaccgagaatctgaacatgttttacctgatcctgaagctgctgaaccacaaagagctgaccaacctgaagggcagcctggaaaagtaccagtccgccaacaaagaagaaaccttcagcgacgagttggaactgatcaacctgctgaacctggacaacaacagagtgaccgaggacttcgagctggaagccaacgagatcggcaagttcctggacttcaacgaaaacaaaatcaaggaccggaaagagctgaaaaagttcgacaccaacaagatctatttcgacggcgagaacatcatcaagcaccgggccttctacaatatcaagaaatacggcatgctgaatctgctggaaaagatcgccgataaggccaagtataagatcagcctgaaagaactgaaagagtacagcaacaagaagaatgagattgaaaagaactacaccatgcagcagaacctgcaccggaagtacgccagacccaagaaggacgaaaagttcaacgacgaggactacaaagagtatgagaaggccatcggcaacatccagaagtacacccacctgaagaacaaggtggaattcaatgagctgaacctgctgcagggcctgctgctgaagatcctgcaccggctcgtgggctacaccagcatctgggagcgggacctgagattccggctgaagggcgagtttcccgagaaccactacatcgaggaaattttcaatttcgacaactccaagaatgtgaagtacaaaagcggccagatcgtggaaaagtatatcaacttctacaaagaactgtacaaggacaatgtggaaaagcggagcatctactccgacaagaaagtgaagaaactgaagcaggagaagaaagacctgtatattgcaaactacatcgctcactttaattatattcctcatgccgagattagcctgctggaagtgctggaaaacctgcggaagctgctgtcctacgaccggaagctgaagaacgccatcatgaagtccatcgtggacattctgaaagaatacggcttcgtggccaccttcaagatcggcgctgacaagaagatcgaaatccagaccctggaatcagagaagatcgtgcacctgaagaatctgaagaaaaagaaactgatgaccgaccggaacagcgaggaactgtgcgaactcgtgaaagtcatgttcgagtacaaggccctggaaggaggaggtggaagcggaggaggaggaagcggaggaggaggtagcgtgagcaagggcgaggagctgttcaccggggtggtgcccatcctggtcgagctggacggcgacgtaaacggccacaagttcagcgtgtccggcgagggcgagggcgatgccacctacggcaagctgaccctgaagttcatctgcaccaccggcaagctgcccgtgccctggcccaccctcgtgaccaccctgacctacggcgtgcagtgcttcagccgctaccccgaccacatgaagcagcacgacttcttcaagtccgccatgcccgaaggctacgtccaggagcgcaccatcttcttcaaggacgacggcaactacaagacccgcgccgaggtgaagttcgagggcgacaccctggtgaaccgcatcgagctgaagggcatcgacttcaaggaggacggcaacatcctggggcacaagctggagtacaactacaacagccacaacgtctatatcatggccgacaagcagaagaacggcatcaaggtgaacttcaagatccgccacaacatcgaggacggcagctgcagctcgccgaccactaccagcagaacacccccatcggcgacggccccgtgctgctgcccgacaaccactacctgagcacccagtccgccctgagcaaagaccccaacgagaagcgcgatcacatggtcctgctggagttcgtgaccgccgccgggatcactctcggcatggacgagctgtactaa

SEQ ID NO: 3 - DNA, 2272 bp, Artificial Sequence
  SASRS-CoV-2.0
tgcatctcaattagtcagcaaccatagtcccgcccctaactccgcccatcccgcccctaactccgcccagttccgcccattctccgccccatcgctgactaattttttttatttatgcagaggccgaggccgcctcggcctctgagctattccagaagtagtgaggaggcttttttggaggcctaggcttttgcaaaaagcttcttcccaggtaacaaaccaaccaactttcgatctcttgtagatctgttctctaaacgaactttaaaatctgtgtggctgtcactcggctgcatgcttagtgcactcacgcagtataattaataactaattactgtcgttgacaggacacgagtaactcgtctatcttctgcaggctgcttacggtttcgtccgtgttgcagccgatcatcagcacatctaggtttcgtccgggtgtgaccgaaaggtaagccaccatggaagacgccaaaaacataaagaaaggcccggcgccattctatccgctggaagatggaaccgctggagagcaactgcataaggctatgaagagatacgccctggttcctggaacaattgcttttacagatgcacatatcgaggtggacatcacttacgctgagtacttcgaaatgtccgttcggttggcagaagctatgaaacgatatgggctgaatacaaatcacagaatcgtcgtatgcagtgaaaactctcttcaattctttatgccggtgttgggcgcgttatttatcggagttgcagttgcgcccgcgaacgacatttataataacgtgaattgctcaacagtatgggcatttcgcagcctaccgtggtgttcgtttccaaaaaggggttgcaaaaaattttgaacgtgcaaaaaaagctcccaatcatccaaaaaattattatcatggattctaaaacggattaccagggatttcagtcgatgtacacgttcgtcacatctcatctacctcccggttttaatgaatacgattttgtgccagagtccttcgatagggacaagacaattgcactgatcatgaactcctctggatctactggtctgcctaaaggtgtcgctctgcctcatagaactgcctgcgtgagattctcgcatgccagagatcctatttttggcaatcaaatcattccggatactgcgattttaagtgttgttccattccatcacggttttggaatgtttactacactcggatatttgatatgtggatttcgagtcgtcttaatgtatagatttgaagaagagctgtttctgaggagccttcaggattacaagattcaaagtgcgctgctggtgccaaccctattctccttcttcgccaaaagcactctgattgacaaatacgatttatctaatttacacgaaattgcttctggtggcgctcccctctctaaggaagtcggggaagcggttgccaagaggttccatctgccaggtatcaggcaaggatatgggctcactgagactacatcagctattctgattacacccgagggggatgataaaccgggcgcggtcggtaaagttgttccattttttgaagcgaaggttgtggatctggataccgggaaaacgctgggcgttaatcaaagaggcgaactgtgtgtgagaggtcctatgattatgtccggttatgtaaacaatccggaagcgaccaacgccttgattgacaaggatggatggctacattctggagacatagcttactgggacgaagacgaacacttcttcatcgttgaccgcctgaagtctctgattaagtacaaaggctatcaggtggctcccgctgaattggaatccatcttgctccaacaccccaacatcttcgacgcaggtgtcgcaggtcttcccgacgatgacgccggtgaacttcccgccgccgttgttgttttggagcacggaaagacgatgacggaaaaagagatcgtggattacgtcgccagtcaagtaacaaccgcgaaaaagttgcgcggaggagttgtgtttgtggacgaagtaccgaaaggtcttaccggaaaactcgacgcaagaaaaatcagagagatcctcataaaggccaagaagggcggaaagatcgccgtgtaattctagagtcggggcggccggccgcttcgagcagacatgataagatacattgatgagtttggacaaaccacaactagaatgcagtgaaaaaaatgctttatttgtgaaatttgtgatgctattgctttatttgtaaccattataagctgcaataaacaagtt

SEQ ID NO: 4 - protein, 164 aa, Artificial Sequence
  Cas13.N.a.a
MKVTKVDGISHKKYIEEGKLVKSTSEENRTSERLSELLSIRLDIYIKNPDNASEEENRIRRENLKKFFSNKVLHLKDSVLYLKNRKEKNAVQDKNYSEEDISEYDLKNKNSFSVLKKILLNEDVNSEELEIFRKDVEAKLNKINSLKYSFEENKANYQKINENN

SEQ ID NO: 5 - protein, 1003 aa, Artificial Sequence
  dCas13.C.a.a
VEKVGGKSKRNIIYDYYRESAKRNDYINNVQEAFDKLYKKEDIEKLFFLIENSKKHEKYKIREYYHKIIGRKNDKENFAKIIYEEIQNVNNIKELIEKIPDMSELKKSQVFYKYYLDKEELNDKNIKYAFCHFVEIEMSQLLKNYVYKRLSNISNDKIKRIFEYQNLKKLIENKLLNKLDTYVRNCGKYNYYLQVGEIATSDFIARNRQNEAFLRNIIGVSSVAYFSLRNILETENENGITGRMRGKTVKNNKGEEKYVSGEVDKIYNENKQNEVKENLKMFYSYDFNMDNKNEIEDFFANIDEAISSIAHGIVHFNLELEGKDIFAFKNIAPSEISKKMFQNEINEKKLKLKIFKQLNSANVFNYYEKDVIIKYLKNTKFNFVNKNIPFVPSFTKLYNKIEDLRNTLKFFWSVPKDKEEKDAQIYLLKNIYYGEFLNKFVKNSKVFFKITNEVIKINKQRNQKTGHYKYQKFENIEKTVPVEYLAIIQSREMINNQDKEEKNTYIDFIQQIFLKGFIDYLNKNNLKYIESNNNNDNNDIFSKIKIKKDNKEKYDKILKNYEKHNRNKEIPHEINEFVREIKLGKILKYTENLNMFYLILKLLNHKELTNLKGSLEKYQSANKEETFSDELELINLLNLDNNRVTEDFELEANEIGKFLDFNENKIKDRKELKKFDTNKIYFDGENIIKHRAFYNIKKYGMLNLLEKIADKAKYKISLKELKEYSNKKNEIEKNYTMQQNLHRKYARPKKDEKFNDEDYKEYEKAIGNIQKYTHLKNKVEFNELNLLQGLLLKILHRLVGYTSIWERDLRFRLKGEFPENHYIEEIFNFDNSKNVKYKSGQIVEKYINFYKELYKDNVEKRSIYSDKKVKKLKQEKKDLYIANYIAHFNYIPHAEISLLEVLENLRKLLSYDRKLKNAIMKSIVDILKEYGFVATFKIGADKKIEIQTLESEKIVHLKNLKKKKLMTDRNSEELCELVKVMFEYKALEGGGGSGGGGSGGGGS

SEQ ID NO: 6 - DNA, 28 bp, Artificial Sequence
  Guide RNA
gggaccgggggttccgcgtctagtttct

SEQ ID NO: 7 - DNA, 28 bp, Artificial Sequence
  Guide RNA
gggaccgggggttccgcgtctagtttct

SEQ ID NO: 8 - DNA, 28 bp, Artificial Sequence
  Guide RNA
ggacagagccctggactggagctggggg

SEQ ID NO: 9 - DNA, 28 bp, Artificial Sequence
  Guide RNA
gagacaggagatcgagaccttcgtgggg

SEQ ID NO: 10 - DNA, 28 bp, Artificial Sequence
  Guide RNA
tgtgaggggacacggtctcgtcacgtct

SEQ ID NO: 11 - DNA, 28 bp, Artificial Sequence
  Guide RNA
ccacgagcagggctggggagaaggtggg

SEQ ID NO: 12 - DNA, 28 bp, Artificial Sequence
  Guide RNA
ccccggtgggtcggggaaggagtggaga

SEQ ID NO: 13 - DNA, 28 bp, Artificial Sequence
  Guide RNA
tgtgttggagaagctgcaggtgaaggtg

SEQ ID NO: 14 - DNA, 28 bp, Artificial Sequence
  Guide RNA
gtcccactgtccacgccggagcctccgg

SEQ ID NO: 15 - DNA, 28 bp, Artificial Sequence
  Guide RNA
gtgcatcttccttctccgagacgtcacc

SEQ ID NO: 16 - DNA, 28 bp, Artificial Sequence
  Guide RNA
cgtcttcgacgtcggagtgcatcttcct

SEQ ID NO: 17 - DNA, 28 bp, Artificial Sequence
  Guide RNA
cgggctccctacactcgtccaccggccc

SEQ ID NO: 18 - DNA, 28 bp, Artificial Sequence
  Guide RNA
ccggcccctccgaaacaccccggtgggt

SEQ ID NO: 19 - DNA, 28 bp, Artificial Sequence
  Guide RNA
aggagtggagagaggtagagagtctgag

SEQ ID NO: 20 - DNA, 28 bp, Artificial Sequence
  Guide RNA
cgcccgtctcgagtcccactgtccacgc

SEQ ID NO: 21 - DNA, 28 bp, Artificial Sequence
  Guide RNA
gcctccggggccccgtccccactcgact

SEQ ID NO: 22 - DNA, 28 bp, Artificial Sequence
  Guide RNA
ctcggccaggaccccacccacaggggag

SEQ ID NO: 23 - DNA, 28 bp, Artificial Sequence
  Guide RNA
caggggaggacgtgtcctagtcctcgag

SEQ ID NO: 24 - DNA, 414 bp, Homo sapiens
cccgaaagtgtgtgtctcctgaggagttcacagaaataatgaaccaaagagagcaattctaccataaggtgaatttctccccacctggtgacacaaacagccttttcccaggtacttggtacctggagcgagtggacgagcagcatcgccgaaagtatgcccggcgtcccgtctaaaggtgttctgcagatccatggaaagcttcctgggaaacgtatgctagcagagcttctccccgtgaatcatatttttaagatcccactcttagctggtaaatgaatttgaatcgacatagtagccccataagcatcagccctgtagagtgaggagccatctctagcgggcccttcattcctctccatgctgcaatcactgtcctgggcttatggtgctatggactaggggtcctttgtg

SEQ ID NO: 25 - DNA, 489 bp, Homo sapiens
gcagtcacagcagagatggaaagctgctaatgatgctggctactttaatgatgaaatggcaccaattgaagtgaagacaaagaaaggaaaacagacaatgcaggtagacgagcatgctcggccccaaaccaccctggaacagttacagaaacttcctccagtattcaagaaagatggaactgttactgcagggaatgcatcgggtgtagctgatggtgctggagctgttatcatagctagtgaagatgctgttaagaaacataacttcacaccactggcaagaattgtgggctactttgtatctggatgtgatccctctatcatgggtattggtcctgtccctgctatcagtggggcactgaagaaagcaggactgagtcttaaggacatggatttggtagaggtgaatgaagcttttgctccccagtacttggctgttgagaggagtttggatcttgacataagtaaaaccaatgtgaatggaggagc